European Patent Application EP 4 775 218 A1, published July 15, 2026. Title: 冠状病毒的3CL蛋白酶用于预防或治疗肿瘤的用途. Applicant: 中国人民解放军军事科学院军事医学研究院. The sequence listing filed with the application follows.

SEQUENCE LISTING (13 sequences)

SEQ ID NO: 1 - RNA, 918 nt, synthetic construct
  source 1..918: mol_type = other RNA
agtggttttagaaaaatggcattcccatctggtaaagttgagggttgtatggtacaagtaacttgtggtacaactacacttaacggtctttggcttgatgacgtagtttactgtccaagacatgtgatctgcacctctgaagacatgcttaaccctaattatgaagatttactcattcgtaagtctaatcataatttcttggtacaggctggtaatgttcaactcagggttattggacattctatgcaaaattgtgtacttaagcttaaggttgatacagccaatcctaagacacctaagtataagtttgttcgcattcaaccaggacagactttttcagtgttagcttgttacaatggttcaccatctggtgtttaccaatgtgctatgaggcccaatttcactattaagggttcattccttaatggttcatgtggtagtgttggttttaacatagattatgactgtgtctctttttgttacatgcaccatatggaattaccaactggagttcatgctggcacagacttagaaggtaacttttatggaccttttgttgacaggcaaacagcacaagcagctggtacggacacaactattacagttaatgttttagcttggttgtacgctgctgttataaatggagacaggtggtttctcaatcgatttaccacaactcttaatgactttaaccttgtggctatgaagtacaattatgaacctctaacacaagaccatgttgacatactaggacctctttctgctcaaactggaattgccgttttagatatgtgtgcttcattaaaagaattactgcaaaatggtatgaatggacgtaccatattgggtagtgctttattagaagatgaatttacaccttttgatgttgttagacaatgctcaggtgttactttccaa

SEQ ID NO: 2 - RNA, 51 nt, synthetic construct
  source 1..51: mol_type = other RNA
gggaaataagagagaaaagaagagtaagaagaaatataagaccccggcgcc

SEQ ID NO: 3 - skipped

SEQ ID NO: 4 - RNA, 111 nt, synthetic construct
  source 1..111: mol_type = other RNA
gctggagcctcggtggcctagcttcttgccccttgggcctccccccagcccctcctccccttcctgcacccgtacccccgtggtctttgaataaagtctgagtgggcggca

SEQ ID NO: 5 - RNA, 110 nt, synthetic construct
  source 1..110: mol_type = other RNA
aaaaaaaaaaaaaaaaaaaaaaaaaaaaaagcatatgactaaaaaaaaaaaaaaaaaaaaaaaaaaaaaaaaaaaaaaaaaaaaaaaaaaaaaaaaaaaaaaaaaaaaaa

SEQ ID NO: 6 - protein, 307 aa, synthetic construct
MSGFRKMAFPSGKVEGCMVQVTCGTTTLNGLWLDDVVYCPRHVICTSEDMLNPNYEDLLIRKSNHNFLVQAGNVQLRVIGHSMQNCVLKLKVDTANPKTPKYKFVRIQPGQTFSVLACYNGSPSGVYQCAMRPNFTIKGSFLNGSCGSVGFNIDYDCVSFCYMHHMELPTGVHAGTDLEGNFYGPFVDRQTAQAAGTDTTITVNVLAWLYAAVINGDRWFLNRFTTTLNDFNLVAMKYNYEPLTQDHVDILGPLSAQTGIAVLDMCASLKELLQNGMNGRTILGSALLEDEFTPFDVVRQCSGVTFQ

SEQ ID NO: 7 - RNA, 1208 nt, synthetic construct
  source 1..1208: mol_type = other RNA
gggaaataagagagaaaagaagagtaagaagaaatataagaccccggcgccgccaccatgagtggttttagaaaaatggcattcccatctggtaaagttgagggttgtatggtacaagtaacttgtggtacaactacacttaacggtctttggcttgatgacgtagtttactgtccaagacatgtgatctgcacctctgaagacatgcttaaccctaattatgaagatttactcattcgtaagtctaatcataatttcttggtacaggctggtaatgttcaactcagggttattggacattctatgcaaaattgtgtacttaagcttaaggttgatacagccaatcctaagacacctaagtataagtttgttcgcattcaaccaggacagactttttcagtgttagcttgttacaatggttcaccatctggtgtttaccaatgtgctatgaggcccaatttcactattaagggttcattccttaatggttcatgtggtagtgttggttttaacatagattatgactgtgtctctttttgttacatgcaccatatggaattaccaactggagttcatgctggcacagacttagaaggtaacttttatggaccttttgttgacaggcaaacagcacaagcagctggtacggacacaactattacagttaatgttttagcttggttgtacgctgctgttataaatggagacaggtggtttctcaatcgatttaccacaactcttaatgactttaaccttgtggctatgaagtacaattatgaacctctaacacaagaccatgttgacatactaggacctctttctgctcaaactggaattgccgttttagatatgtgtgcttcattaaaagaattactgcaaaatggtatgaatggacgtaccatattgggtagtgctttattagaagatgaatttacaccttttgatgttgttagacaatgctcaggtgttactttccaatgataataggctggagcctcggtggcctagcttcttgccccttgggcctccccccagcccctcctccccttcctgcacccgtacccccgtggtctttgaataaagtctgagtgggcggcaaaaaaaaaaaaaaaaaaaaaaaaaaaaaaagcatatgactaaaaaaaaaaaaaaaaaaaaaaaaaaaaaaaaaaaaaaaaaaaaaaaaaaaaaaaaaaaaaaaaaaaaaa

SEQ ID NO: 8 - RNA, 891 nt, synthetic construct
  source 1..891: mol_type = other RNA
aggaaaatggcattcccgtcaggcaaagttgaagggtgcatggtacaagtaacctgtggaactacaactcttaatggattgtggttggatgacacagtatactgtccaagacatgtcatttgcacagcagaagacatgcttaatcctaactatgaagatctgctcattcgcaaatccaaccatagctttcttgttcaggctggcaatgttcaacttcgtgttattggccattctatgcaaaattgtctgcttaggcttaaagttgatacttctaaccctaagacacccaagtataaatttgtccgtatccaacctggtcaaacattttcagttctagcatgctacaatggttcaccatctggtgtttatcagtgtgccatgagacctaatcataccattaaaggttctttccttaatggatcatgtggtagtgttggttttaacattgattatgattgcgtgtctttctgctatatgcatcatatggagcttccaacaggagtacacgctggtactgacttagaaggtaaattctatggtccatttgttgacagacaaactgcacaggctgcaggtacagacacaaccataaccttaaatgttttggcatggctgtatgctgctgttatcaatggtgataggtggtttcttaatagattcaccactactttgaatgactttaaccttgtggcaatgaagtacaactatgaacctttgacacaagatcatgttgacatattgggacctctttctgctcaaacaggaattgccgtcttagatatgtgtgctgctttgaaagagctgctgcagaatggtatgaatggtcgtactatccttggtagcactattttagaagatgagtttacaccatttgatgttgttagacaatgc

SEQ ID NO: 9 - RNA, 1181 nt, synthetic construct
  source 1..1181: mol_type = other RNA
gggaaataagagagaaaagaagagtaagaagaaatataagaccccggcgccgccaccatgaggaaaatggcattcccgtcaggcaaagttgaagggtgcatggtacaagtaacctgtggaactacaactcttaatggattgtggttggatgacacagtatactgtccaagacatgtcatttgcacagcagaagacatgcttaatcctaactatgaagatctgctcattcgcaaatccaaccatagctttcttgttcaggctggcaatgttcaacttcgtgttattggccattctatgcaaaattgtctgcttaggcttaaagttgatacttctaaccctaagacacccaagtataaatttgtccgtatccaacctggtcaaacattttcagttctagcatgctacaatggttcaccatctggtgtttatcagtgtgccatgagacctaatcataccattaaaggttctttccttaatggatcatgtggtagtgttggttttaacattgattatgattgcgtgtctttctgctatatgcatcatatggagcttccaacaggagtacacgctggtactgacttagaaggtaaattctatggtccatttgttgacagacaaactgcacaggctgcaggtacagacacaaccataaccttaaatgttttggcatggctgtatgctgctgttatcaatggtgataggtggtttcttaatagattcaccactactttgaatgactttaaccttgtggcaatgaagtacaactatgaacctttgacacaagatcatgttgacatattgggacctctttctgctcaaacaggaattgccgtcttagatatgtgtgctgctttgaaagagctgctgcagaatggtatgaatggtcgtactatccttggtagcactattttagaagatgagtttacaccatttgatgttgttagacaatgctgataataggctggagcctcggtggcctagcttcttgccccttgggcctccccccagcccctcctccccttcctgcacccgtacccccgtggtctttgaataaagtctgagtgggcggcaaaaaaaaaaaaaaaaaaaaaaaaaaaaaaagcatatgactaaaaaaaaaaaaaaaaaaaaaaaaaaaaaaaaaaaaaaaaaaaaaaaaaaaaaaaaaaaaaaaaaaaaaa

SEQ ID NO: 10 - protein, 298 aa, synthetic construct
MRKMAFPSGKVEGCMVQVTCGTTTLNGLWLDDTVYCPRHVICTAEDMLNPNYEDLLIRKSNHSFLVQAGNVQLRVIGHSMQNCLLRLKVDTSNPKTPKYKFVRIQPGQTFSVLACYNGSPSGVYQCAMRPNHTIKGSFLNGSCGSVGFNIDYDCVSFCYMHHMELPTGVHAGTDLEGKFYGPFVDRQTAQAAGTDTTITLNVLAWLYAAVINGDRWFLNRFTTTLNDFNLVAMKYNYEPLTQDHVDILGPLSAQTGIAVLDMCAALKELLQNGMNGRTILGSTILEDEFTPFDVVRQC

SEQ ID NO: 11 - RNA, 891 nt, synthetic construct
  source 1..891: mol_type = other RNA
gtgaaaatgtcacatcccagtggagatgttgaggcttgtatggttcaggttacctgcggtagcatgactcttaatggtctttggcttgacaacacagtctggtgcccacgacacgtaatgtgcccggctgaccagttgtctgatcctaattatgatgccttgttgatttctatgactaatcatagtttcagtgtgcaaaaacacattggcgctccagcaaacttgcgtgttgttggtcatgccatgcaaggcactcttttgaagttgactgtcgatgttgctaaccctagcactccagcctacacttttacaacagtgaaacctggcgcagcatttagtgtgttagcatgctataatggtcgtccgactggtacattcactgttgtaatgcgccctaactacacaattaagggttcctttctgtgtggttcttgtggtagtgttggttacaccaaggggggtagtgtgatcaatttttgttacatgcatcaaatggaacttgctaatggtacacataccggttcagcatttgatggtactatgtatggtgcctttatggataaacaagtgcaccaagttcagttaacagacaaatactgcagtgttaatgtagtagcttggctttacgcagcaatacttaatggttgcgcttggtttgtaaaacctaatcgcactagtgttgtttcttttaatgaatgggctcttgccaaccaattcactgaatttgttggcactcaatccgttgacatgttagctgtcaaaacaggcgttgctattgaacagctgctttatgcgatccaacaactttatactgggttccagggaaagcaaatccttggcagtaccatgttggaagatgaattcacacctgaggatgttaatatgcagatt

SEQ ID NO: 12 - RNA, 1181 nt, synthetic construct
  source 1..1181: mol_type = other RNA
gggaaataagagagaaaagaagagtaagaagaaatataagaccccggcgccgccaccatggtgaaaatgtcacatcccagtggagatgttgaggcttgtatggttcaggttacctgcggtagcatgactcttaatggtctttggcttgacaacacagtctggtgcccacgacacgtaatgtgcccggctgaccagttgtctgatcctaattatgatgccttgttgatttctatgactaatcatagtttcagtgtgcaaaaacacattggcgctccagcaaacttgcgtgttgttggtcatgccatgcaaggcactcttttgaagttgactgtcgatgttgctaaccctagcactccagcctacacttttacaacagtgaaacctggcgcagcatttagtgtgttagcatgctataatggtcgtccgactggtacattcactgttgtaatgcgccctaactacacaattaagggttcctttctgtgtggttcttgtggtagtgttggttacaccaaggggggtagtgtgatcaatttttgttacatgcatcaaatggaacttgctaatggtacacataccggttcagcatttgatggtactatgtatggtgcctttatggataaacaagtgcaccaagttcagttaacagacaaatactgcagtgttaatgtagtagcttggctttacgcagcaatacttaatggttgcgcttggtttgtaaaacctaatcgcactagtgttgtttcttttaatgaatgggctcttgccaaccaattcactgaatttgttggcactcaatccgttgacatgttagctgtcaaaacaggcgttgctattgaacagctgctttatgcgatccaacaactttatactgggttccagggaaagcaaatccttggcagtaccatgttggaagatgaattcacacctgaggatgttaatatgcagatttgataataggctggagcctcggtggcctagcttcttgccccttgggcctccccccagcccctcctccccttcctgcacccgtacccccgtggtctttgaataaagtctgagtgggcggcaaaaaaaaaaaaaaaaaaaaaaaaaaaaaaagcatatgactaaaaaaaaaaaaaaaaaaaaaaaaaaaaaaaaaaaaaaaaaaaaaaaaaaaaaaaaaaaaaaaaaaaaaa

SEQ ID NO: 13 - protein, 298 aa, synthetic construct
MVKMSHPSGDVEACMVQVTCGSMTLNGLWLDNTVWCPRHVMCPADQLSDPNYDALLISMTNHSFSVQKHIGAPANLRVVGHAMQGTLLKLTVDVANPSTPAYTFTTVKPGAAFSVLACYNGRPTGTFTVVMRPNYTIKGSFLCGSCGSVGYTKGGSVINFCYMHQMELANGTHTGSAFDGTMYGAFMDKQVHQVQLTDKYCSVNVVAWLYAAILNGCAWFVKPNRTSVVSFNEWALANQFTEFVGTQSVDMLAVKTGVAIEQLLYAIQQLYTGFQGKQILGSTMLEDEFTPEDVNMQI